European Patent Specification EP 4 225 803 B1, published April 15, 2026. Title: Nanoparticle for Anti-Cancer Peptides and Uses Thereof. Applicant: King's College London Academia Sinica. The sequence listing filed with the application follows.

SEQUENCE LISTING (39 sequences)

SEQ ID NO: 1 - protein, 14 aa, Artificial Sequence
  DEE
GLLDLLELLLEAAG

SEQ ID NO: 2 - protein, 14 aa, Artificial Sequence
  EEE
GLLELLELLLEAAG

SEQ ID NO: 3 - protein, 14 aa, Artificial Sequence
  HEE
GLLHLLELLLEAAG

SEQ ID NO: 4 - protein, 14 aa, Artificial Sequence
  KEE
GLLKLLELLLEAAG

SEQ ID NO: 5 - protein, 14 aa, Artificial Sequence
  DHE
GLLDLLHLLLEAAG

SEQ ID NO: 6 - protein, 14 aa, Artificial Sequence
  EHE
GLLELLHLLLEAAG

SEQ ID NO: 7 - protein, 14 aa, Artificial Sequence
  HHE
GLLHLLHLLLEAAG

SEQ ID NO: 8 - protein, 14 aa, Artificial Sequence
  KHE
GLLKLLHLLLEAAG

SEQ ID NO: 9 - protein, 14 aa, Artificial Sequence
  DKE
GLLDLLKLLLEAAG

SEQ ID NO: 10 - protein, 14 aa, Artificial Sequence
  EKE
GLLELLKLLLEAAG

SEQ ID NO: 11 - protein, 14 aa, Artificial Sequence
  HKE
GLLHLLKLLLEAAG

SEQ ID NO: 12 - protein, 14 aa, Artificial Sequence
  KKE
GLLKLLKLLLEAAG

SEQ ID NO: 13 - protein, 14 aa, Artificial Sequence
  DEH
GLLDLLELLLHAAG

SEQ ID NO: 14 - protein, 14 aa, Artificial Sequence
  EEH
GLLELLELLLHAAG

SEQ ID NO: 15 - protein, 14 aa, Artificial Sequence
  HEH
GLLHLLELLLHAAG

SEQ ID NO: 16 - protein, 14 aa, Artificial Sequence
  KEH
GLLKLLELLLHAAG

SEQ ID NO: 17 - protein, 14 aa, Artificial Sequence
  DHH
GLLDLLHLLLHAAG

SEQ ID NO: 18 - protein, 14 aa, Artificial Sequence
  EHH
GLLELLHLLLHAAG

SEQ ID NO: 19 - protein, 14 aa, Artificial Sequence
  HHH
GLLHLLHLLLHAAG

SEQ ID NO: 20 - protein, 14 aa, Artificial Sequence
  KHH
GLLKLLHLLLHAAG

SEQ ID NO: 21 - protein, 14 aa, Artificial Sequence
  DKH
GLLDLLKLLLHAAG

SEQ ID NO: 22 - protein, 14 aa, Artificial Sequence
  EKH
GLLELLKLLLHAAG

SEQ ID NO: 23 - protein, 14 aa, Artificial Sequence
  HKH
GLLHLLKLLLHAAG

SEQ ID NO: 24 - protein, 14 aa, Artificial Sequence
  KKH
GLLKLLKLLLHAAG

SEQ ID NO: 25 - protein, 14 aa, Artificial Sequence
  DEK
GLLDLLELLLKAAG

SEQ ID NO: 26 - protein, 14 aa, Artificial Sequence
  EEK
GLLELLELLLKAAG

SEQ ID NO: 27 - protein, 14 aa, Artificial Sequence
  HEK
GLLHLLELLLKAAG

SEQ ID NO: 28 - protein, 14 aa, Artificial Sequence
  KEK
GLLKLLELLLKAAG

SEQ ID NO: 29 - protein, 14 aa, Artificial Sequence
  DHK
GLLDLLHLLLKAAG

SEQ ID NO: 30 - protein, 14 aa, Artificial Sequence
  EHK
GLLELLHLLLKAAG

SEQ ID NO: 31 - protein, 14 aa, Artificial Sequence
  HHK
GLLHLLHLLLKAAG

SEQ ID NO: 32 - protein, 14 aa, Artificial Sequence
  KHK
GLLKLLHLLLKAAG

SEQ ID NO: 33 - protein, 14 aa, Artificial Sequence
  DKK
GLLDLLKLLLKAAG

SEQ ID NO: 34 - protein, 14 aa, Artificial Sequence
  EKK
GLLELLKLLLKAAG

SEQ ID NO: 35 - protein, 14 aa, Artificial Sequence
  HKK
GLLHLLKLLLKAAG

SEQ ID NO: 36 - protein, 14 aa, Artificial Sequence
  KKK
GLLKLLKLLLKAAG

SEQ ID NO: 37 - protein, 14 aa, Artificial Sequence
  25B2
GLDDLAKLLLKLAG

SEQ ID NO: 38 - protein, 14 aa, Artificial Sequence
  GLLxLLxLLLxAAG
  MISC_FEATURE (4)..(4): X is selected from arginine (R), histidine (H), lysine (K), aspartic acid (D) or glutamic acid (E)
  MISC_FEATURE (7)..(7): X is selected from arginine (R), histidine (H), lysine (K), aspartic acid (D) or glutamic acid (E)
  MISC_FEATURE (11)..(11): X is selected from arginine (R), histidine (H), lysine (K), aspartic acid (D) or glutamic acid (E)
GLLXLLXLLLXAAG

SEQ ID NO: 39 - protein, 14 aa, Artificial Sequence
  GLLxLLELLLxAAG
  MISC_FEATURE (4)..(4): X is selected from arginine (R), histidine (H), lysine (K), aspartic acid (D) or glutamic acid (E)
  MISC_FEATURE (11)..(11): X is selected from arginine (R), histidine (H), lysine (K), aspartic acid (D) or glutamic acid (E)
GLLXLLELLLXAAG